European Patent Application EP 4 119 573 A1, published January 18, 2023. Title: RECOMBINANT HUMAN TYPE XVII COLLAGEN, AND PREPARATION METHOD AND USE THEREOF. Applicant: JIANGSU TRAUTEC MEDICAL TECHNOLOGY CO., LTD. The sequence listing filed with the application follows.

SEQUENCE LISTING (10 sequences)

SEQ ID NO: 1 - protein, 1497 aa, Homo sapiens
MDVTKKNKRDGTEVTERIVTETVTTRLTSLPPKGGTSNGYAKTASLGGGSRLEKQSLTHGSSGYINSTGSTRGHASTSSYRRAHSPASTLPNSPGSTFERKTHVTRHAYEGSSSGNSSPEYPRKEFASSSTRGRSQTRESEIRVRLQSASPSTRWTELDDVKRLLKGSRSASVSPTRNSSNTLPIPKKGTVETKIVTASSQSVSGTYDATILDANLPSHVWSSTLPAGSSMGTYHNNMTTQSSSLLNTNAYSAGSVFGVPNNMASCSPTLHPGLSTSSSVFGMQNNLAPSLTTLSHGTTTTSTAYGVKKNMPQSPAAVNTGVSTSAACTTSVQSDDLLHKDCKFLILEKDNTPAKKEMELLIMTKDSGKVFTASPASIAATSFSEDTLKKEKQAAYNADSGLKAEANGDLKTVSTKGKTTTADIHSYGSSGGGGSGGGGGVGGAGGGPWGPAPAWCPCGSCCSWWKWLLGLLLTWLLLLGLLFGLIALAEEVRKLKARVDELERIRRSILPYGDSMDRIEKDRLQGMAPAAGADLDKIGLHSDSQEELWMFVRKKLMMEQENGNLRGSPGPKGDMGSPGPKGDRGFPGTPGIPGPLGHPGPQGPKGQKGSVGDPGMEGPMGQRGREGPMGPRGEAGPPGSGEKGERGAAGEPGPHGPPGVPGSVGPKGSSGSPGPQGPPGPVGLQGLRGEVGLPGVKGDKGPMGPPGPKGDQGEKGPRGLTGEPGMRGLPGAVGEPGAKGAMGPAGPDGHQGPRGEQGLTGMPGIRGPPGPSGDPGKPGLTGPQGPQGLPGTPGRPGIKGEPGAPGKIVTSEGSSMLTVPGPPGPPGAMGPPGPPGAPGPAGPAGLPGHQEVLNLQGPPGPPGPRGPPGPSIPGPPGPRGPPGEGLPGPPGPPGSFLSNSETFLSGPPGPPGPPGPKGDQGPPGPRGHQGEQGLPGFSTSGSSSFGLNLQGPPGPPGPQGPKGDKGDPGVPGALGIPSGPSEGGSSSTMYVSGPPGPPGPPGPPGSISSSGQEIQQYISEYMQSDSIRSYLSGVQGPPGPPGPPGPVTTITGETFDYSELASHVVSYLRTSGYGVSLFSSSISSEDILAVLQRDDVRQYLRQYLMGPRGPPGPPGASGDGSLLSLDYAELSSRILSYMSSSGISIGLPGPPGPPGLPGTSYEELLSLLRGSEFRGIVGPPGPPGPPGIPGNVWSSISVEDLSSYLHTAGLSFIPGPPGPPGPPGPRGPPGVSGALATYAAENSDSFRSELISYLTSPDVRSFIVGPPGPPGPQGPPGDSRLLSTDASHSRGSSSSSHSSSVRRGSSYSSSMSTGGGGAGSLGAGGAFGEAAGDRGPYGTDIGPGGGYGAAAEGGMYAGNGGLLGADFAGDLDYNELAVRVSESMQRQGLLQGMAYTVQGPPGQPGPQGPPGISKVFSAYSNVTADLMDFFQTYGAIQGPPGQKGEMGTPGPKGDRGPAGPPGHPGPPGPRGHKGEKGDKGDQVYAGRRRRRSIAVKP

SEQ ID NO: 2 - protein, 233 aa, Artificial Sequence
GSPGPKGDMGSPGPKGDRGFPGTPGIPGPLGHPGPQGPKGQKGSVGDPGMEGPGEKGERGAAGEPGPHGPPGVPGSVGPKGSSGSPGPQGPPGPVGLQGLRGEVGLPGVKGDKGPMGPPGPKGDQGEKGPPGPPGPPGPKGDQGPPGPRGHQGEQGLPGFSGPPGPPGPQGPKGDKGDPGVPGALGIPGPPGQKGEMGTPGPKGDRGPAGPPGHPGPPGPRGHKGEKGDKGDQ

SEQ ID NO: 3 - protein, 466 aa, Artificial Sequence
GSPGPKGDMGSPGPKGDRGFPGTPGIPGPLGHPGPQGPKGQKGSVGDPGMEGPGEKGERGAAGEPGPHGPPGVPGSVGPKGSSGSPGPQGPPGPVGLQGLRGEVGLPGVKGDKGPMGPPGPKGDQGEKGPPGPPGPPGPKGDQGPPGPRGHQGEQGLPGFSGPPGPPGPQGPKGDKGDPGVPGALGIPGPPGQKGEMGTPGPKGDRGPAGPPGHPGPPGPRGHKGEKGDKGDQGSPGPKGDMGSPGPKGDRGFPGTPGIPGPLGHPGPQGPKGQKGSVGDPGMEGPGEKGERGAAGEPGPHGPPGVPGSVGPKGSSGSPGPQGPPGPVGLQGLRGEVGLPGVKGDKGPMGPPGPKGDQGEKGPPGPPGPPGPKGDQGPPGPRGHQGEQGLPGFSGPPGPPGPQGPKGDKGDPGVPGALGIPGPPGQKGEMGTPGPKGDRGPAGPPGHPGPPGPRGHKGEKGDKGDQ

SEQ ID NO: 4 - protein, 249 aa, Artificial Sequence
YVWSHPQFEKGSPGPKGDMGSPGPKGDRGFPGTPGIPGPLGHPGPQGPKGQKGSVGDPGMEGPGEKGERGAAGEPGPHGPPGVPGSVGPKGSSGSPGPQGPPGPVGLQGLRGEVGLPGVKGDKGPMGPPGPKGDQGEKGPPGPPGPPGPKGDQGPPGPRGHQGEQGLPGFSGPPGPPGPQGPKGDKGDPGVPGALGIPGPPGQKGEMGTPGPKGDRGPAGPPGHPGPPGPRGHKGEKGDKGDQHHHHHH

SEQ ID NO: 5 - protein, 482 aa, Artificial Sequence
YVWSHPQFEKGSPGPKGDMGSPGPKGDRGFPGTPGIPGPLGHPGPQGPKGQKGSVGDPGMEGPGEKGERGAAGEPGPHGPPGVPGSVGPKGSSGSPGPQGPPGPVGLQGLRGEVGLPGVKGDKGPMGPPGPKGDQGEKGPPGPPGPPGPKGDQGPPGPRGHQGEQGLPGFSGPPGPPGPQGPKGDKGDPGVPGALGIPGPPGQKGEMGTPGPKGDRGPAGPPGHPGPPGPRGHKGEKGDKGDQGSPGPKGDMGSPGPKGDRGFPGTPGIPGPLGHPGPQGPKGQKGSVGDPGMEGPGEKGERGAAGEPGPHGPPGVPGSVGPKGSSGSPGPQGPPGPVGLQGLRGEVGLPGVKGDKGPMGPPGPKGDQGEKGPPGPPGPPGPKGDQGPPGPRGHQGEQGLPGFSGPPGPPGPQGPKGDKGDPGVPGALGIPGPPGQKGEMGTPGPKGDRGPAGPPGHPGPPGPRGHKGEKGDKGDQHHHHHH

SEQ ID NO: 6 - DNA, 699 bp, Artificial Sequence
ggttctcctggtccaaaaggtgacatgggttctccaggtcctaaaggtgacagaggttttcctggtactccaggtattcctggtccattgggtcatccaggtcctcaaggtccaaaaggtcaaaagggttctgttggtgaccctggtatggaaggtccaggtgaaaagggtgaaagaggtgctgctggtgaacctggtccacacggtccacctggtgttccaggttctgttggtcctaagggttcttctggttctcctggtccacaaggtcctcctggtccagttggtttgcaaggtttgagaggtgaagttggtttgccaggtgttaagggtgacaagggtccaatgggtcctccaggtccaaaaggtgaccaaggtgaaaagggtccacctggtcctcctggtccacctggtccaaagggtgaccaaggtcctccaggtcctagaggtcatcaaggtgaacaaggtttgcctggtttttctggtccaccaggtcctccaggtccacaaggtcctaaaggtgacaaaggtgacccaggtgttcctggtgctttgggtattccaggtccacctggtcaaaaaggtgaaatgggtactccaggtcctaagggtgacagaggtccagctggtccacctggtcatcctggtccaccaggtccaagaggtcataagggtgaaaaaggtgacaagggtgaccaa

SEQ ID NO: 7 - DNA, 1398 bp, Artificial Sequence
ggttctccaggtcctaaaggtgacatgggttctccaggtcctaagggtgacagaggttttccaggtactccaggtattccaggtcctttgggtcatccaggtcctcaaggtcctaaaggtcaaaaaggttctgttggtgaccctggtatggaaggtcctggtgaaaaaggtgaaagaggtgctgctggtgaacctggtccacacggtcctccaggtgttcctggttctgttggtccaaaaggttcttctggttctcctggtccacaaggtcctccaggtcctgttggtttgcaaggtttgagaggtgaagttggtttgccaggtgttaaaggtgacaaaggtccaatgggtcctccaggtccaaagggtgaccaaggtgaaaaaggtccacctggtcctcctggtccaccaggtccaaaaggtgaccaaggtccacctggtccaagaggtcaccaaggtgaacaaggtttgcctggtttttctggtcctccaggtcctcctggtcctcaaggtccaaagggtgacaagggtgaccctggtgttccaggtgctttgggtattcctggtcctccaggtcaaaagggtgagatgggtactcctggtcctaagggtgacagaggtccagctggtcctcctggtcacccaggtcctcctggtcctagaggtcataaaggtgaaaaaggtgacaagggtgaccaaggttctccaggtccaaagggtgacatgggttctcctggtccaaaaggtgacagaggtttccctggtactccaggtattcctggtccattgggtcacccaggtccacaaggtccaaaaggtcaaaaaggttctgttggtgacccaggtatggaaggtccaggtgaaaagggtgaaagaggtgctgctggtgaaccaggtcctcatggtccaccaggtgttccaggttctgttggtccaaagggttcttctggttctccaggtccacaaggtcctccaggtccagttggtttgcaaggtttgagaggtgaagttggtttgcctggtgttaagggtgacaaaggtcctatgggtcctcctggtcctaaaggtgaccaaggtgaaaagggtccaccaggtcctccaggtccacctggtccaaaaggtgaccaaggtccaccaggtcctagaggtcatcaaggtgaacaaggtttgccaggtttttctggtccaccaggtccaccaggtcctcaaggtcctaagggtgacaaaggtgacccaggtgttcctggtgctttgggtattcctggtccacctggtcaaaagggtgaaatgggtactcctggtcctaaaggtgacagaggtcctgctggtccacctggtcatccaggtccacctggtccaagaggtcacaaaggtgaaaagggtgacaagggtgaccaa

SEQ ID NO: 8 - DNA, 758 bp, Artificial Sequence
tacgtatggtctcatccacaattcgagaagggttctcctggtccaaaaggtgacatgggttctccaggtcctaaaggtgacagaggttttcctggtactccaggtattcctggtccattgggtcatccaggtcctcaaggtccaaaaggtcaaaagggttctgttggtgaccctggtatggaaggtccaggtgaaaagggtgaaagaggtgctgctggtgaacctggtccacacggtccacctggtgttccaggttctgttggtcctaagggttcttctggttctcctggtccacaaggtcctcctggtccagttggtttgcaaggtttgagaggtgaagttggtttgccaggtgttaagggtgacaagggtccaatgggtcctccaggtccaaaaggtgaccaaggtgaaaagggtccacctggtcctcctggtccacctggtccaaagggtgaccaaggtcctccaggtcctagaggtcatcaaggtgaacaaggtttgcctggtttttctggtccaccaggtcctccaggtccacaaggtcctaaaggtgacaaaggtgacccaggtgttcctggtgctttgggtattccaggtccacctggtcaaaaaggtgaaatgggtactccaggtcctaagggtgacagaggtccagctggtccacctggtcatcctggtccaccaggtccaagaggtcataagggtgaaaaaggtgacaagggtgaccaacaccatcatcaccatcattaagcggccgc

SEQ ID NO: 9 - DNA, 1457 bp, Artificial Sequence
tacgtatggtctcatcctcaatttgaaaagggttctccaggtcctaaaggtgacatgggttctccaggtcctaagggtgacagaggttttccaggtactccaggtattccaggtcctttgggtcatccaggtcctcaaggtcctaaaggtcaaaaaggttctgttggtgaccctggtatggaaggtcctggtgaaaaaggtgaaagaggtgctgctggtgaacctggtccacacggtcctccaggtgttcctggttctgttggtccaaaaggttcttctggttctcctggtccacaaggtcctccaggtcctgttggtttgcaaggtttgagaggtgaagttggtttgccaggtgttaaaggtgacaaaggtccaatgggtcctccaggtccaaagggtgaccaaggtgaaaaaggtccacctggtcctcctggtccaccaggtccaaaaggtgaccaaggtccacctggtccaagaggtcaccaaggtgaacaaggtttgcctggtttttctggtcctccaggtcctcctggtcctcaaggtccaaagggtgacaagggtgaccctggtgttccaggtgctttgggtattcctggtcctccaggtcaaaagggtgagatgggtactcctggtcctaagggtgacagaggtccagctggtcctcctggtcacccaggtcctcctggtcctagaggtcataaaggtgaaaaaggtgacaagggtgaccaaggttctccaggtccaaagggtgacatgggttctcctggtccaaaaggtgacagaggtttccctggtactccaggtattcctggtccattgggtcacccaggtccacaaggtccaaaaggtcaaaaaggttctgttggtgacccaggtatggaaggtccaggtgaaaagggtgaaagaggtgctgctggtgaaccaggtcctcatggtccaccaggtgttccaggttctgttggtccaaagggttcttctggttctccaggtccacaaggtcctccaggtccagttggtttgcaaggtttgagaggtgaagttggtttgcctggtgttaagggtgacaaaggtcctatgggtcctcctggtcctaaaggtgaccaaggtgaaaagggtccaccaggtcctccaggtccacctggtccaaaaggtgaccaaggtccaccaggtcctagaggtcatcaaggtgaacaaggtttgccaggtttttctggtccaccaggtccaccaggtcctcaaggtcctaagggtgacaaaggtgacccaggtgttcctggtgctttgggtattcctggtccacctggtcaaaagggtgaaatgggtactcctggtcctaaaggtgacagaggtcctgctggtccacctggtcatccaggtccacctggtccaagaggtcacaaaggtgaaaagggtgacaagggtgaccaacaccatcaccatcatcattaagcggccgc

SEQ ID NO: 10 - DNA, 4550 bp, Artificial Sequence
gaattctggagtcatcctcaattcgaaaaaatggatgtcactaaaaagaacaagagagacggaactgaggtcactgagagaatcgttaccgaaactgtcaccacaagacttacttcattacctccaaagggtggaacttctaatggttacgcaaagacagcatcattaggaggtggttcaagacttgagaaacaatcccttactcatggttcaagtggatacataaattcaactggttcaacaagaggacatgcaagtacttcttcttatagaagagcacatagtccagcatcaactttgcccaactctcctggttcaacatttgagagaaaaactcatgtaaccagacatgcctatgagggttctagttctggtaattcatctccagaataccctagaaaagagtttgcatcatcctcaactagaggtagatcacagactagagaatctgaaatcagagtcagattacaatcagcatctccttcaactagatggactgagttagacgacgtgaaaagattattaaagggatcaagaagtgcaagtgtttcccctacaagaaattcttccaacacccttcccattcctaagaaaggaaccgttgaaactaaaatcgttacagcatcatctcagtctgtatccggaacctacgacgctaccattctggacgccaacttaccttctcatgtctggtcttcaactttacccgcaggttcctcaatgggaacttaccacaataacatgactactcaatcaagttctcttctgaataccaatgcatactcagccggttccgtttttggagtccctaacaatatggcctcttgctccccaactcttcatccaggtctttcaacctcatcaagtgtatttggtatgcagaacaacttagccccttccttgacaaccctgtctcatggtactactaccactagtacagcatatggagtcaagaagaacatgccacagtcacctgctgccgttaacactggagtttcaacatctgctgcctgcactacatctgttcaatcagatgatcttctgcataaggactgcaagtttttaattttagagaaagacaatacccctgccaaaaaggaaatggagttacttataatgaccaaagattctggtaaagtattcactgcttctcccgctagtatcgccgcaacttcattctctgaagatactttaaagaaggaaaaacaagccgcatacaacgcagactcaggtttaaaagcagaagcaaacggtgaccttaaaacagtgtcaactaagggaaagactacaaccgcagacatccattcatatggttcttcaggtggaggaggatctggaggaggtggtggagtgggaggtgctggaggaggtccatggggtcctgcacctgcatggtgcccttgcggttcttgctgcagttggtggaagtggcttctgggtttattattaacttggctgcttttactgggtcttttattcggtcttatcgcattagcagaagaggtcagaaaacttaaggccagagttgatgagttagagagaatcagaagatcaatccttccctatggagactccatggacagaatcgaaaaggatagacttcagggtatggcccctgcagcaggagctgatctggataaaatcggacttcattcagattctcaagaggaattatggatgtttgttagaaagaaacttatgatggagcaggagaacggtaacctgagaggttctcctggtccaaaaggagatatgggttcacccggtcccaaaggagatagaggattccctggtactccaggtatccccggtcccctgggtcaccctggacctcaaggtcctaaaggtcaaaagggttctgtaggagatccaggtatggagggtcccatgggtcagagaggtagagaaggtcccatgggaccaagaggtgaagctggacctcccggaagtggtgaaaaaggagaaagaggagcagcaggagaacctggaccccatggacctccaggagttcctggatcagtcggacccaaaggttcatccggttctcctggacctcaaggtccaccaggacccgtcggattgcaaggattgagaggagaagttggacttcccggagttaagggtgacaagggtcctatgggtcctcctggtccaaagggagatcagggtgaaaagggtcctagaggtctgactggtgaaccaggaatgagaggacttcccggtgccgtgggtgaacccggtgcaaaaggagcaatgggtcctgccggtcctgatggacaccagggacccagaggagagcagggattaacaggaatgcctggtatcagaggtcccccaggtccctcaggagacccaggaaagccaggacttactggtccccagggtcctcaaggtctgcctggaactcccggaagacccggaatcaaaggtgaaccaggagccccaggaaaaatcgttactagtgaaggatcttcaatgctgactgtgccaggtccacctggtcctcctggagctatgggtcctcccggtccccctggagcacccggtcctgcaggtcctgccggattacctggacatcaggaagtcttaaacctgcaaggtccaccaggtcctcctggtccaagaggaccccctggtccttcaatccctggtccacctggacctagaggtccacccggagagggacttcccggaccaccaggacctcctggatcatttctgtctaattctgagacatttctttcaggacctcctggtcctcccggaccacctggaccaaaaggagatcagggaccacctggtcccagaggacatcaaggagagcagggtcttccaggtttctctacttctggatcatcatcatttggtcttaatcttcaaggtcctcctggacccccaggaccacagggacccaagggtgacaagggagaccctggagtcccaggtgcactgggaatcccttcaggtccttcagaaggtggttcatcttcaaccatgtatgtgtctggacccccaggacctcccggacctccaggtcctcctggttcaatctcttcttctggtcaagaaattcagcagtatatttctgagtacatgcaatctgactctattagaagttatttgtctggtgtgcagggtccaccaggtcctccaggtccccctggaccagtcactactatcactggagagacatttgattatagtgaattagcatcacacgtcgtttcttatctgagaacttcaggttatggtgtttcattattttcctcctcaatctcttcagaagacatcttagccgtactgcagagagatgatgtaagacagtaccttagacaatacttgatgggtccaagaggaccaccaggtccacccggtgcatcaggagacggatcattattatctttggattacgctgaattatcatcaagaatccttagttacatgtcctcttctggtatctccataggtctgcccggtcctcctggtcctcccggacttcctggtacttcttacgaagagcttctgtcacttttaagaggatctgagtttagaggtatagttggtcccccaggacctccaggtcctccaggtatcccaggtaacgtgtggtcatctatctcagttgaggatctttcatcttatcttcacaccgccggattgtcctttatacctggtcctccaggaccccctggacctcctggacccagaggtcctccaggagtatccggtgctttagcaacttatgcagcagaaaactccgattcttttagatcagaattgatctcctaccttacttctcctgatgttagatcattcatcgtcggacctccaggaccacctggacctcaaggacctcctggagattcaagattactgagtacagatgcatcacattcaagaggttcaagttcttcttctcactcctcttctgttagaagaggatcatcatattcatcaagtatgtcaactggtggaggaggagctggttcattgggtgccggaggtgcatttggtgaggccgctggtgacagaggaccttatggtactgacattggacctggtggaggttatggtgcagcagcagaaggtggaatgtatgctggtaatggaggtttactgggagccgactttgccggagacctggactacaacgagttagctgttagagtgtcagagtcaatgcagagacaaggattattacagggtatggcttatacagttcagggacccccaggtcagccaggtcctcaaggaccccctggtatttcaaaagtcttctccgcttattctaacgttactgcagacctgatggatttcttccagacttacggtgccatccaaggtcctccaggacagaagggtgaaatgggaactcccggtcccaagggtgacagaggtcctgcaggacctcctggtcaccctggaccacctggacctagaggacacaaaggtgagaagggtgacaagggagaccaggtttacgcaggaagaagaagaagaagaagtattgccgtcaagcctcaccatcaccatcatcactaagcggccgc